European Patent Application EP 4 775 691 A2, published July 15, 2026. Title: MODULATION OF GENE EXPRESSION AND SCREENING FOR DEREGULATED PROTEIN EXPRESSION. Applicant: UNIVERSITY OF SOUTHAMPTON. The sequence listing filed with the application follows.

SEQUENCE LISTING (127 sequences)

SEQ ID NO: 1 - DNA, 31 bp, synthetic construct
  misc_feature 1..31: note = Description of Artificial Sequence: Synthetic primer
  source 1..31: mol_type = other DNA
ataaagcttcttgttataaggttttgattcc

SEQ ID NO: 2 - DNA, 31 bp, synthetic construct
  misc_feature 1..31: note = Description of Artificial Sequence: Synthetic primer
  source 1..31: mol_type = other DNA
atatctagatgtacataccctgaaaagtcac

SEQ ID NO: 3 - DNA, 19 bp, synthetic construct
  misc_feature 1..19: note = Description of Artificial Sequence: Synthetic primer
  source 1..19: mol_type = other DNA
agtcgaggctgatcagcgg

SEQ ID NO: 4 - DNA, 26 bp, synthetic construct
  misc_feature 1..26: note = Description of Artificial Sequence: Synthetic primer
  source 1..26: mol_type = other DNA
gagggtaccagagacagtgggatggc

SEQ ID NO: 5 - DNA, 21 bp, synthetic construct
  misc_feature 1..21: note = Description of Artificial Sequence: Synthetic primer
  source 1..21: mol_type = other DNA
ggctcatgtaacgtcatcaat

SEQ ID NO: 6 - DNA, 35 bp, synthetic construct
  misc_feature 1..35: note = Description of Artificial Sequence: Synthetic primer
  source 1..35: mol_type = other DNA
atacaatttaccataatttacttttgaattatgtt

SEQ ID NO: 7 - DNA, 33 bp, synthetic construct
  misc_feature 1..33: note = Description of Artificial Sequence: Synthetic primer
  source 1..33: mol_type = other DNA
aagtaaattatggtaaattgtatcatacattag

SEQ ID NO: 8 - DNA, 37 bp, synthetic construct
  misc_feature 1..37: note = Description of Artificial Sequence: Synthetic primer
  source 1..37: mol_type = other DNA
ccttgccagaccagtttcctagttatctatattgaac

SEQ ID NO: 9 - DNA, 32 bp, synthetic construct
  misc_feature 1..32: note = Description of Artificial Sequence: Synthetic primer
  source 1..32: mol_type = other DNA
taactaggaaactggtctggcaaggtggctta

SEQ ID NO: 10 - DNA, 31 bp, synthetic construct
  misc_feature 1..31: note = Description of Artificial Sequence: Synthetic primer
  source 1..31: mol_type = other DNA
cttcaagggaccttggccgggtgcggtggct

SEQ ID NO: 11 - DNA, 33 bp, synthetic construct
  misc_feature 1..33: note = Description of Artificial Sequence: Synthetic primer
  source 1..33: mol_type = other DNA
gcacccggccaaggtcccttgaagtttatctaa

SEQ ID NO: 12 - DNA, 39 bp, synthetic construct
  misc_feature 1..39: note = Description of Artificial Sequence: Synthetic primer
  source 1..39: mol_type = other DNA
acacaaacaaagcttaggtttctttcttgtcaccttcta

SEQ ID NO: 13 - DNA, 38 bp, synthetic construct
  misc_feature 1..38: note = Description of Artificial Sequence: Synthetic primer
  source 1..38: mol_type = other DNA
agaaagaaacctaagctttgtttgtgtgttttatacaa

SEQ ID NO: 14 - DNA, 36 bp, synthetic construct
  misc_feature 1..36: note = Description of Artificial Sequence: Synthetic primer
  source 1..36: mol_type = other DNA
tgcctcatttacgtcatacaacttaatgatagacct

SEQ ID NO: 15 - DNA, 32 bp, synthetic construct
  misc_feature 1..32: note = Description of Artificial Sequence: Synthetic primer
  source 1..32: mol_type = other DNA
ttaagttgtatgacgtaaatgaggcagggcaa

SEQ ID NO: 16 - DNA, 37 bp, synthetic construct
  misc_feature 1..37: note = Description of Artificial Sequence: Synthetic primer
  source 1..37: mol_type = other DNA
tgatacaatttacctcatacaacttaatgatagacct

SEQ ID NO: 17 - DNA, 36 bp, synthetic construct
  misc_feature 1..36: note = Description of Artificial Sequence: Synthetic primer
  source 1..36: mol_type = other DNA
attaagttgtatgaggtaaattgtatcatacattag

SEQ ID NO: 18 - RNA, 19 nt, synthetic construct
  misc_feature 1..19: note = Description of Artificial Sequence: Synthetic primer
  source 1..19: mol_type = other RNA
aacttaaaggttatatctc

SEQ ID NO: 19 - RNA, 20 nt, synthetic construct
  misc_feature 1..20: note = Description of Artificial Sequence: Synthetic primer
  source 1..20: mol_type = other RNA
tataaatacgaataaatcga

SEQ ID NO: 20 - RNA, 19 nt, synthetic construct
  misc_feature 1..19: note = Description of Artificial Sequence: Synthetic primer
  source 1..19: mol_type = other RNA
catgggttggctatgctag

SEQ ID NO: 21 - RNA, 18 nt, synthetic construct
  misc_feature 1..18: note = Description of Artificial Sequence: Synthetic primer
  source 1..18: mol_type = other RNA
caacacgacataaccaaa

SEQ ID NO: 22 - RNA, 20 nt, synthetic construct
  misc_feature 1..20: note = Description of Artificial Sequence: Synthetic primer
  source 1..20: mol_type = other RNA
aagccaatcagagggagaca

SEQ ID NO: 23 - RNA, 23 nt, synthetic construct
  misc_feature 1..23: note = Description of Artificial Sequence: Synthetic primer
  source 1..23: mol_type = other RNA
aacatttctatttagttaaaagc

SEQ ID NO: 24 - RNA, 20 nt, synthetic construct
  misc_feature 1..20: note = Description of Artificial Sequence: Synthetic primer
  source 1..20: mol_type = other RNA
tcgtgtattacaacagttaa

SEQ ID NO: 25 - RNA, 18 nt, synthetic construct
  misc_feature 1..18: note = Description of Artificial Sequence: Synthetic primer
  source 1..18: mol_type = other RNA
caaccagtttgcattcgt

SEQ ID NO: 26 - RNA, 19 nt, synthetic construct
  misc_feature 1..19: note = Description of Artificial Sequence: Synthetic primer
  source 1..19: mol_type = other RNA
ttagtattccttgacttta

SEQ ID NO: 27 - RNA, 23 nt, synthetic construct
  misc_feature 1..23: note = Description of Artificial Sequence: Synthetic primer
  source 1..23: mol_type = other RNA
ttctgtacactgtttagtattcc

SEQ ID NO: 28 - RNA, 18 nt, synthetic construct
  misc_feature 1..18: note = Description of Artificial Sequence: Synthetic primer
  source 1..18: mol_type = other RNA
gaagagggagtgaaggtt

SEQ ID NO: 29 - RNA, 18 nt, synthetic construct
  misc_feature 1..18: note = Description of Artificial Sequence: Synthetic primer
  source 1..18: mol_type = other RNA
aaagcttggtgagattga

SEQ ID NO: 30 - RNA, 23 nt, synthetic construct
  misc_feature 1..23: note = Description of Artificial Sequence: Synthetic primer
  source 1..23: mol_type = other RNA
tttcttgaaaagtggaaagcttg

SEQ ID NO: 31 - RNA, 24 nt, synthetic construct
  misc_feature 1..24: note = Description of Artificial Sequence: Synthetic primer
  source 1..24: mol_type = other RNA
tggaatgagggacggttgtttttc

SEQ ID NO: 32 - RNA, 18 nt, synthetic construct
  misc_feature 1..18: note = Description of Artificial Sequence: Synthetic primer
  source 1..18: mol_type = other RNA
ggtatgagaactatagga

SEQ ID NO: 33 - RNA, 18 nt, synthetic construct
  misc_feature 1..18: note = Description of Artificial Sequence: Synthetic primer
  source 1..18: mol_type = other RNA
aaacaaacagcagggtat

SEQ ID NO: 34 - RNA, 18 nt, synthetic construct
  misc_feature 1..18: note = Description of Artificial Sequence: Synthetic primer
  source 1..18: mol_type = other RNA
ggtaataagtgtcacaaa

SEQ ID NO: 35 - RNA, 18 nt, synthetic construct
  misc_feature 1..18: note = Description of Artificial Sequence: Synthetic primer
  source 1..18: mol_type = other RNA
gtatcatacattagaagg

SEQ ID NO: 36 - RNA, 20 nt, synthetic construct
  misc_feature 1..20: note = Description of Artificial Sequence: Synthetic primer
  source 1..20: mol_type = other RNA
tcaaaagtaaattatggtct

SEQ ID NO: 37 - RNA, 25 nt, synthetic construct
  misc_feature 1..25: note = Description of Artificial Sequence: Synthetic primer
  source 1..25: mol_type = other RNA
gactggtaaataataaacataattc

SEQ ID NO: 38 - RNA, 21 nt, synthetic construct
  misc_feature 1..21: note = Description of Artificial Sequence: Synthetic primer
  source 1..21: mol_type = other RNA
aaatgtatactggagaagact

SEQ ID NO: 39 - RNA, 22 nt, synthetic construct
  misc_feature 1..22: note = Description of Artificial Sequence: Synthetic primer
  source 1..22: mol_type = other RNA
atatattagagatacatcagcc

SEQ ID NO: 40 - RNA, 24 nt, synthetic construct
  misc_feature 1..24: note = Description of Artificial Sequence: Synthetic primer
  source 1..24: mol_type = other RNA
gacaaacatttaatgaatactcaa

SEQ ID NO: 41 - RNA, 24 nt, synthetic construct
  misc_feature 1..24: note = Description of Artificial Sequence: Synthetic primer
  source 1..24: mol_type = other RNA
ttgactccttcttttgacaaacat

SEQ ID NO: 42 - RNA, 19 nt, synthetic construct
  misc_feature 1..19: note = Description of Artificial Sequence: Synthetic primer
  source 1..19: mol_type = other RNA
tttaaatccttccttactt

SEQ ID NO: 43 - RNA, 20 nt, synthetic construct
  misc_feature 1..20: note = Description of Artificial Sequence: Synthetic primer
  source 1..20: mol_type = other RNA
gattataaaacaaacgaagc

SEQ ID NO: 44 - RNA, 23 nt, synthetic construct
  misc_feature 1..23: note = Description of Artificial Sequence: Synthetic primer
  source 1..23: mol_type = other RNA
tgttttaatataagttgcttcaa

SEQ ID NO: 45 - RNA, 19 nt, synthetic construct
  misc_feature 1..19: note = Description of Artificial Sequence: Synthetic primer
  source 1..19: mol_type = other RNA
tgtggggtgaccacagctt

SEQ ID NO: 46 - RNA, 18 nt, synthetic construct
  misc_feature 1..18: note = Description of Artificial Sequence: Synthetic primer
  source 1..18: mol_type = other RNA
tcccttacttatatccaa

SEQ ID NO: 47 - RNA, 19 nt, synthetic construct
  misc_feature 1..19: note = Description of Artificial Sequence: Synthetic primer
  source 1..19: mol_type = other RNA
ccaagtttggttacttatc

SEQ ID NO: 48 - RNA, 21 nt, synthetic construct
  misc_feature 1..21: note = Description of Artificial Sequence: Synthetic primer
  source 1..21: mol_type = other RNA
gaagtttatctaatattgacc

SEQ ID NO: 49 - RNA, 22 nt, synthetic construct
  misc_feature 1..22: note = Description of Artificial Sequence: Synthetic primer
  source 1..22: mol_type = other RNA
ggtctatcattaagttgtatga

SEQ ID NO: 50 - RNA, 21 nt, synthetic construct
  misc_feature 1..21: note = Description of Artificial Sequence: Synthetic primer
  source 1..21: mol_type = other RNA
ttaaataagacttcaggtcta

SEQ ID NO: 51 - RNA, 24 nt, synthetic construct
  misc_feature 1..24: note = Description of Artificial Sequence: Synthetic primer
  source 1..24: mol_type = other RNA
ttagagaatcattttaaataagac

SEQ ID NO: 52 - RNA, 24 nt, synthetic construct
  misc_feature 1..24: note = Description of Artificial Sequence: Synthetic primer
  source 1..24: mol_type = other RNA
cttaatccaattcttcaattttag

SEQ ID NO: 53 - RNA, 25 nt, synthetic construct
  misc_feature 1..25: note = Description of Artificial Sequence: Synthetic oligonucleotide
  source 1..25: mol_type = other RNA
cttctatgcagccaacctgtagact

SEQ ID NO: 54 - RNA, 24 nt, synthetic construct
  misc_feature 1..24: note = Description of Artificial Sequence: Synthetic oligonucleotide
  source 1..24: mol_type = other RNA
acctttttcttctatgcagccaac

SEQ ID NO: 55 - RNA, 33 nt, synthetic construct
  misc_feature 1..33: note = Description of Artificial Sequence: Synthetic oligonucleotide
  source 1..33: mol_type = other RNA
acctttttcttctatgcagccaacctgtagact

SEQ ID NO: 56 - RNA, 17 nt, synthetic construct
  misc_feature 1..17: note = Description of Artificial Sequence: Synthetic oligonucleotide
  source 1..17: mol_type = other RNA
ctgtaaaagaaaataga

SEQ ID NO: 57 - DNA, 29 bp, synthetic construct
  misc_feature 1..29: note = Description of Artificial Sequence: Synthetic oligonucleotide
  source 1..29: mol_type = other DNA
tctacaggttggctgcatagaagaaaaag

SEQ ID NO: 58 - DNA, 37 bp, synthetic construct
  misc_feature 1..37: note = Description of Artificial Sequence: Synthetic oligonucleotide
  source 1..37: mol_type = other DNA
agtctacaggttggctgcatagaagaaaaaggtagag

SEQ ID NO: 59 - DNA, 41 bp, synthetic construct
  misc_feature 1..41: note = Description of Artificial Sequence: Synthetic oligonucleotide
  source 1..41: mol_type = other DNA
tcttagtctacaggttggctgcatagaagaaaaaggtagag

SEQ ID NO: 60 - DNA, 41 bp, synthetic construct
  misc_feature 1..41: note = Description of Artificial Sequence: Synthetic oligonucleotide
  source 1..41: mol_type = other DNA
tctcagtctacaggttggctgcatagaagaaaaaggtagag

SEQ ID NO: 61 - DNA, 24 bp, synthetic construct
  misc_feature 1..24: note = Description of Artificial Sequence: Synthetic oligonucleotide
  source 1..24: mol_type = other DNA
tcatcgaatacttttggaaataag

SEQ ID NO: 62 - DNA, 38 bp, synthetic construct
  misc_feature 1..38: note = Description of Artificial Sequence: Synthetic oligonucleotide
  source 1..38: mol_type = other DNA
tagtctacaggttggctgcatagaagaaaaaggtagag

SEQ ID NO: 63 - DNA, 20 bp, synthetic construct
  misc_feature 1..20: note = Description of Artificial Sequence: Synthetic oligonucleotide
  source 1..20: mol_type = other DNA
cctctcagtctacaggttgg

SEQ ID NO: 64 - DNA, 20 bp, synthetic construct
  misc_feature 1..20: note = Description of Artificial Sequence: Synthetic oligonucleotide
  source 1..20: mol_type = other DNA
cctcttagtctacaggttgg

SEQ ID NO: 65 - DNA, 59 bp, synthetic construct
  misc_feature 1..59: note = Description of Artificial Sequence: Synthetic oligonucleotide
  source 1..59: mol_type = other DNA
gtagagttatttataatcttgtaaatcttggactttgagtcatctattttcttttacgg

SEQ ID NO: 66 - DNA, 42 bp, synthetic construct
  misc_feature 1..42: note = Description of Artificial Sequence: Synthetic oligonucleotide
  source 1..42: mol_type = other DNA
gtagagttatttataatcttgtaaatcttggactttgagtca

SEQ ID NO: 67 - DNA, 79 bp, synthetic construct
  misc_feature 1..79: note = Description of Artificial Sequence: Synthetic oligonucleotide
  source 1..79: mol_type = other DNA
gtagagttatttataattcttgacgttcacagatatacttgtaaatcttggactttgagtcatctattttcttttacag

SEQ ID NO: 68 - DNA, 33 bp, synthetic construct
  misc_feature 1..33: note = Description of Artificial Sequence: Synthetic oligonucleotide
  source 1..33: mol_type = other DNA
gttcagtttttttcttagaaatggaatccgagg

SEQ ID NO: 69 - DNA, 36 bp, synthetic construct
  misc_feature 1..36: note = Description of Artificial Sequence: Synthetic oligonucleotide
  source 1..36: mol_type = other DNA
cttagtctacaggttggctgcatagaagaaaaaggt

SEQ ID NO: 70 - RNA, 470 nt, synthetic construct
  misc_feature 1..470: note = Description of Artificial Sequence: Synthetic polynucleotide
  source 1..470: mol_type = other RNA
ttgtataaaacacacaaacaaagcaaggaaagaatgaagcaacaaagccagagatttactgaaaatgaaattatactccacagagtgggagtgggccctgagcaagtggctcaagggcctggttacagaattttctggggtttaaatacccttcagaggttttccattggttacttggtatacaccctatgtaaatgaagtagtggtctgtaatcagtctgattggttataggaggggaccaatcagaggtacaccctatgtaaatgaagtagtggtctgtaatcagtctgattggttattcaatttcttatctgccacagtaaaagggagggggttgcaaagggagtagcctcttgtccttttgttacttgagcatggaaagttggggttttccttttgatttcgttctaggaggtcagcatggattgaccttaggttccctgcctccagaccttattgccctgcctca

SEQ ID NO: 71 - RNA, 471 nt, synthetic construct
  misc_feature 1..471: note = Description of Artificial Sequence: Synthetic polynucleotide
  source 1..471: mol_type = other RNA
ttggacaaaacgcacaaacaaagcaaggaaagaatgaagcaacaaaagcagagatttattgaaaacgaaagtacactccacagggtgggagcgggcccgagcaagcggctcaagggcccggttacagaattttctggggtttaaataccctctagaggtttcccattggttacttggtgtacaccctatgtaaatgaagtagtggcccgcaatcagtctgattggttgcggaaagcgaccaatcagaggtacactcctatgcaaatgaagacttggcccgcgaccagtctgattggttgttcaatttcccatctgccacgcagaaaaggtggggggttgcaaagggagtagcctctggtccttttgttacttgggcgtggaaagttggggttttcctttcgatttagttctaggaagtcagcgtgaatcggccttaggttccctgcctccagaccctattctcctgcctca

SEQ ID NO: 72 - DNA, 26 bp, synthetic construct
  misc_feature 1..26: note = Description of Artificial Sequence: Synthetic primer
  source 1..26: mol_type = other DNA
gagggtaccagagacagtgggatggc

SEQ ID NO: 73 - DNA, 21 bp, synthetic construct
  misc_feature 1..21: note = Description of Artificial Sequence: Synthetic primer
  source 1..21: mol_type = other DNA
ggctcatgtaacgtcatcaat

SEQ ID NO: 74 - DNA, 19 bp, synthetic construct
  misc_feature 1..19: note = Description of Artificial Sequence: Synthetic primer
  source 1..19: mol_type = other DNA
gggagacccaagctggcta

SEQ ID NO: 75 - DNA, 20 bp, synthetic construct
  misc_feature 1..20: note = Description of Artificial Sequence: Synthetic primer
  source 1..20: mol_type = other DNA
agacccagctctcaatgttg

SEQ ID NO: 76 - DNA, 20 bp, synthetic construct
  misc_feature 1..20: note = Description of Artificial Sequence: Synthetic primer
  source 1..20: mol_type = other DNA
tagcttctttcaggcgttta

SEQ ID NO: 77 - DNA, 18 bp, synthetic construct
  misc_feature 1..18: note = Description of Artificial Sequence: Synthetic primer
  source 1..18: mol_type = other DNA
agtggtggggaataaacg

SEQ ID NO: 78 - DNA, 19 bp, synthetic construct
  misc_feature 1..19: note = Description of Artificial Sequence: Synthetic primer
  source 1..19: mol_type = other DNA
cagcagtccacagcacggt

SEQ ID NO: 79 - DNA, 20 bp, synthetic construct
  misc_feature 1..20: note = Description of Artificial Sequence: Synthetic primer
  source 1..20: mol_type = other DNA
ctcagtccagcaggcgtgtg

SEQ ID NO: 80 - DNA, 20 bp, synthetic construct
  misc_feature 1..20: note = Description of Artificial Sequence: Synthetic primer
  source 1..20: mol_type = other DNA
ggtctctgggcaaaggcttc

SEQ ID NO: 81 - DNA, 20 bp, synthetic construct
  misc_feature 1..20: note = Description of Artificial Sequence: Synthetic primer
  source 1..20: mol_type = other DNA
cagaagctgttgggatgtag

SEQ ID NO: 82 - DNA, 20 bp, synthetic construct
  misc_feature 1..20: note = Description of Artificial Sequence: Synthetic primer
  source 1..20: mol_type = other DNA
tctccatcgagaaggtccac

SEQ ID NO: 83 - DNA, 20 bp, synthetic construct
  misc_feature 1..20: note = Description of Artificial Sequence: Synthetic primer
  source 1..20: mol_type = other DNA
tggctcaggacccagtttta

SEQ ID NO: 84 - DNA, 20 bp, synthetic construct
  misc_feature 1..20: note = Description of Artificial Sequence: Synthetic primer
  source 1..20: mol_type = other DNA
tcttctgcctggtcttctcc

SEQ ID NO: 85 - DNA, 19 bp, synthetic construct
  misc_feature 1..19: note = Description of Artificial Sequence: Synthetic primer
  source 1..19: mol_type = other DNA
cctggcttggttcgctacc

SEQ ID NO: 86 - DNA, 20 bp, synthetic construct
  misc_feature 1..20: note = Description of Artificial Sequence: Synthetic primer
  source 1..20: mol_type = other DNA
tgcttcacctgctggtaaaa

SEQ ID NO: 87 - DNA, 21 bp, synthetic construct
  misc_feature 1..21: note = Description of Artificial Sequence: Synthetic primer
  source 1..21: mol_type = other DNA
gaagaacatgcgatatacaca

SEQ ID NO: 88 - DNA, 21 bp, synthetic construct
  misc_feature 1..21: note = Description of Artificial Sequence: Synthetic primer
  source 1..21: mol_type = other DNA
gtctaaaaccaagtcccctat

SEQ ID NO: 89 - DNA, 20 bp, synthetic construct
  misc_feature 1..20: note = Description of Artificial Sequence: Synthetic primer
  source 1..20: mol_type = other DNA
gagggaagatggcggacgag

SEQ ID NO: 90 - DNA, 20 bp, synthetic construct
  misc_feature 1..20: note = Description of Artificial Sequence: Synthetic primer
  source 1..20: mol_type = other DNA
tcctccttggtccgggtgat

SEQ ID NO: 91 - DNA, 20 bp, synthetic construct
  misc_feature 1..20: note = Description of Artificial Sequence: Synthetic primer
  source 1..20: mol_type = other DNA
gcagcggcaaaagtagtaga

SEQ ID NO: 92 - DNA, 19 bp, synthetic construct
  misc_feature 1..19: note = Description of Artificial Sequence: Synthetic primer
  source 1..19: mol_type = other DNA
gtcttgttgctgggttcca

SEQ ID NO: 93 - DNA, 20 bp, synthetic construct
  misc_feature 1..20: note = Description of Artificial Sequence: Synthetic primer
  source 1..20: mol_type = other DNA
aaaatcatcaaaacagcgag

SEQ ID NO: 94 - DNA, 20 bp, synthetic construct
  misc_feature 1..20: note = Description of Artificial Sequence: Synthetic primer
  source 1..20: mol_type = other DNA
tggagcaagtcgcagtttag

SEQ ID NO: 95 - DNA, 20 bp, synthetic construct
  misc_feature 1..20: note = Description of Artificial Sequence: Synthetic primer
  source 1..20: mol_type = other DNA
ggcgacagaaaggttatgaa

SEQ ID NO: 96 - DNA, 20 bp, synthetic construct
  misc_feature 1..20: note = Description of Artificial Sequence: Synthetic primer
  source 1..20: mol_type = other DNA
cgccacaggtcacgtataat

SEQ ID NO: 97 - DNA, 34 bp, synthetic construct
  misc_feature 1..34: note = Description of Artificial Sequence: Synthetic primer
  source 1..34: mol_type = other DNA
atagaattctcgaggggagggttttattctacta

SEQ ID NO: 98 - DNA, 35 bp, synthetic construct
  misc_feature 1..35: note = Description of Artificial Sequence: Synthetic primer
  source 1..35: mol_type = other DNA
atagggccctctagactgtggggagactatggtaa

SEQ ID NO: 99 - DNA, 29 bp, synthetic construct
  misc_feature 1..29: note = Description of Artificial Sequence: Synthetic primer
  source 1..29: mol_type = other DNA
attagaattctctcgggagtcggatgttg

SEQ ID NO: 100 - DNA, 33 bp, synthetic construct
  misc_feature 1..33: note = Description of Artificial Sequence: Synthetic primer
  source 1..33: mol_type = other DNA
attagcggccgcggtacatttctttcgtgttca

SEQ ID NO: 101 - RNA, 25 nt, synthetic construct
  misc_feature 1..25: note = Description of Artificial Sequence: Synthetic oligonucleotide
  source 1..25: mol_type = other RNA
cttctatgcagccaacctgtagact

SEQ ID NO: 102 - RNA, 24 nt, synthetic construct
  misc_feature 1..24: note = Description of Artificial Sequence: Synthetic oligonucleotide
  source 1..24: mol_type = other RNA
acctttttcttctatgcagccaac

SEQ ID NO: 103 - RNA, 24 nt, synthetic construct
  misc_feature 1..24: note = Description of Artificial Sequence: Synthetic oligonucleotide
  source 1..24: mol_type = other RNA
atttccaaaagtattcgatgactg

SEQ ID NO: 104 - RNA, 24 nt, synthetic construct
  misc_feature 1..24: note = Description of Artificial Sequence: Synthetic oligonucleotide
  source 1..24: mol_type = other RNA
tatattaccttatttccaaaagta

SEQ ID NO: 105 - RNA, 25 nt, synthetic construct
  misc_feature 1..25: note = Description of Artificial Sequence: Synthetic oligonucleotide
  source 1..25: mol_type = other RNA
ctgtaaaagaaaatagatgactcaa

SEQ ID NO: 106 - RNA, 17 nt, synthetic construct
  misc_feature 1..17: note = Description of Artificial Sequence: Synthetic oligonucleotide
  source 1..17: mol_type = other RNA
ctgtaaaagaaaataga

SEQ ID NO: 107 - RNA, 25 nt, synthetic construct
  misc_feature 1..25: note = Description of Artificial Sequence: Synthetic oligonucleotide
  source 1..25: mol_type = other RNA
acttacaattccaaaacaatataat

SEQ ID NO: 108 - RNA, 16 nt, synthetic construct
  misc_feature 1..16: note = Description of Artificial Sequence: Synthetic oligonucleotide
  source 1..16: mol_type = other RNA
aggtgctcgcgggtgg

SEQ ID NO: 109 - RNA, 13 nt, synthetic construct
  misc_feature 1..13: note = Description of Artificial Sequence: Synthetic oligonucleotide
  source 1..13: mol_type = other RNA
agttgcttcatct

SEQ ID NO: 110 - RNA, 19 nt, synthetic construct
  misc_feature 1..19: note = Description of Artificial Sequence: Synthetic oligonucleotide
  source 1..19: mol_type = other RNA
ggctgtgattgacttgaat

SEQ ID NO: 111 - RNA, 19 nt, synthetic construct
  misc_feature 1..19: note = Description of Artificial Sequence: Synthetic oligonucleotide
  source 1..19: mol_type = other RNA
gcaagtacgggcttgtcaa

SEQ ID NO: 112 - RNA, 19 nt, synthetic construct
  misc_feature 1..19: note = Description of Artificial Sequence: Synthetic oligonucleotide
  source 1..19: mol_type = other RNA
ggatctactgtcatttgta

SEQ ID NO: 113 - RNA, 19 nt, synthetic construct
  misc_feature 1..19: note = Description of Artificial Sequence: Synthetic oligonucleotide
  source 1..19: mol_type = other RNA
gcagatgaactcggtgatg

SEQ ID NO: 114 - RNA, 21 nt, synthetic construct
  misc_feature 1..21: note = Description of Artificial Sequence: Synthetic oligonucleotide
  source 1..21: mol_type = other RNA
aagatgcagttccgctccatt

SEQ ID NO: 115 - DNA, 117 bp, synthetic construct
  misc_feature 1..117: note = Description of Artificial Sequence: Synthetic polynucleotide
  source 1..117: mol_type = other DNA
cagtctacaggttggctgcatagaagaaaaaggtagagttatttataatcttgtaaatcttggactttgagtcatctattttcttttacagtcatcgaatacttttggaaataaggt

SEQ ID NO: 116 - DNA, 117 bp, synthetic construct
  misc_feature 1..117: note = Description of Artificial Sequence: Synthetic polynucleotide
  source 1..117: mol_type = other DNA
cggtctacaggttggctgcatagaagaaaaaggtagagttatttataatcttgtaaatcttggactttgagtcatctattttcttttacagtcatcgaatacttttggaaataaggt

SEQ ID NO: 117 - DNA, 137 bp, synthetic construct
  misc_feature 1..137: note = Description of Artificial Sequence: Synthetic polynucleotide
  source 1..137: mol_type = other DNA
cggtctacaggttggctgcatagaagaaaaaggtagagttatttataattcttgacgttcacagatatacttgtaaatcttggactttgagtcatctattttcttttacagtcatcgaatacttttggaaataaggt

SEQ ID NO: 118 - DNA, 141 bp, synthetic construct
  misc_feature 1..141: note = Description of Artificial Sequence: Synthetic polynucleotide
  source 1..141: mol_type = other DNA
  misc_feature 1..103: note = DNA
  misc_feature 104..127: note = RNA
  misc_feature 128..141: note = DNA
cagtctacaggttggctgcatagaagaaaaaggtagagttatttataatcttgtaaatcttggactttgagtcatctattttcttttacagtcatcgaatactgggcacagatgaagcaacttgccctttggaaataaggt

SEQ ID NO: 119 - DNA, 161 bp, synthetic construct
  misc_feature 1..161: note = Description of Artificial Sequence: Synthetic polynucleotide
  source 1..161: mol_type = other DNA
  misc_feature 1..123: note = DNA
  misc_feature 124..147: note = RNA
  misc_feature 148..161: note = DNA
cagtctacaggttggctgcatagaagaaaaaggtagagttatttataattcttgacgttcacagatatacttgtaaatcttggactttgagtcatctattttcttttacagtcatcgaatactgggcacagatgaagcaacttgccctttggaaataaggt

SEQ ID NO: 120 - protein, 6 aa, synthetic construct
  REGION 1..6: note = Description of Artificial Sequence: Synthetic peptide
  VARIANT 1..6: note = D-Arg or L-Arg
RRRRRR

SEQ ID NO: 121 - protein, 7 aa, synthetic construct
  REGION 1..7: note = Description of Artificial Sequence: Synthetic peptide
PKKKRKV

SEQ ID NO: 122 - protein, 12 aa, synthetic construct
  REGION 1..12: note = Description of Artificial Sequence: Synthetic peptide
  UNSURE 2
  UNSURE 5
  UNSURE 8
  UNSURE 11
RXRRXRRXRRXR

SEQ ID NO: 123 - protein, 12 aa, synthetic construct
  REGION 1..12: note = Description of Artificial Sequence: Synthetic peptide
  UNSURE 11
  MOD_RES 12: note = Beta-Ala
RFFRFFRFFRXA

SEQ ID NO: 124 - protein, 10 aa, synthetic construct
  REGION 1..10: note = Description of Artificial Sequence: Synthetic peptide
KFFKFFKFFK

SEQ ID NO: 125 - protein, 15 aa, synthetic construct
  REGION 1..15: note = Description of Artificial Sequence: Synthetic peptide
  VARIANT 1..15: note = D-Arg or L-Arg
RRRRRRRRRRRRRRR

SEQ ID NO: 126 - protein, 9 aa, synthetic construct
  REGION 1..9: note = Description of Artificial Sequence: Synthetic peptide
  VARIANT 1..9: note = D-Arg or L-Arg
RRRRRRRRR

SEQ ID NO: 127 - DNA, 38 bp, synthetic construct
  misc_feature 1..38: note = Description of Artificial Sequence: Synthetic oligonucleotide
  source 1..38: mol_type = other DNA
actgttcagtttttttcttagaaatggaatccgaggat